European Patent Specification EP 3 930 849 B1, published February 19, 2025. Title: Protein Secretion Inhibitors. Applicant: Kezar Life Sciences. The sequence listing filed with the application follows.

SEQUENCE LISTING (2 sequences)

SEQ ID NO: 1 - protein, 30 aa, Artificial Sequence
  Synthetic Polypeptide
MQIPQAPWPVVWAVLQLGWRPGWFLDSPDR

SEQ ID NO: 2 - protein, 23 aa, Artificial Sequence
  Synthetic Polypeptide
MRANDALQVLGLLFSLARGSEVG